European Patent Application EP 4 112 738 A1, published January 4, 2023. Title: MULTIGENE ANALYSIS OF TUMOR SAMPLES. Applicant: FOUNDATION MEDICINE, INC. The sequence listing filed with the application follows.

SEQUENCE LISTING (3 sequences)

SEQ ID NO: 1 - DNA, 150 bp, Artificial Sequence
  Description of Artificial Sequence: Synthetic polynucleotide
  modified_base (16)..(135): a, c, t, g, unknown or other
atcgcaccagcgtgtnnnnnnnnnnnnnnnnnnnnnnnnnnnnnnnnnnnnnnnnnnnnnnnnnnnnnnnnnnnnnnnnnnnnnnnnnnnnnnnnnnnnnnnnnnnnnnnnnnnnnnnnnnnnnnnnnnnnnnnncactgcggctcctca

SEQ ID NO: 2 - DNA, 23 bp, Artificial Sequence
  Description of Artificial Sequence: Synthetic primer
aatgatacggcgaccaccgagat

SEQ ID NO: 3 - DNA, 21 bp, Artificial Sequence
  Description of Artificial Sequence: Synthetic primer
caagcagaagacggcatacga